European Patent Specification EP 4 022 047 B1, published April 22, 2026. Title: IMPROVED POLYPEPTIDES CAPABLE OF CONVERTING SUBSTRATE 3-KETO- DEOXYNIVALENOL INTO 3-EPI- DEOXYNIVALENOL. Applicant: Erber Aktiengesellschaft. The sequence listing filed with the application follows.

SEQUENCE LISTING (101 sequences)

SEQ ID NO: 1 - protein, 353 aa, Artificial Sequence
  Enzyme
MDYRYLGRSGLRVSVLTMGTMTFGGSEKVGHTAQADATRQIDLCLDHGINLLDTANVYNAGVSEEMIGVALSEHGRRQKALIATKVRFRMGNGPNEVGLSRHHIIAQAEASLKRLKTDVIDLYQVHEWDGMTPIEETMEALDTLVKQGKVRYVGCSNYSGWHIMKALAAADKHHGQRFISQQIHYTLHSREAEYELVPISQDQGLGILIWSPLAGGLLSGKYRRDGGPDAGRHVGGFREPPVYDWDKLYDIIDVIVAIARERDVSGAQVALAWALGRPGVTSAIIGGRSEAQFRDNLAAAELKLTDDERARLDAASRPPLLYPYWHQSFTAQDRLDQIDLDLIGPYAEEFKRG

SEQ ID NO: 2 - protein, 353 aa, Artificial Sequence
  Enzyme
MDYRYLGRSGLKVSSLTMGTMTFGGSEKVGHTPQAEATRQIDLCLDHGINLLDTANVYNAGVSEEMIGVALAENGRRQKALVATKVRFRMGDGPNEVGLSRHHIVAQAEASLKRLKTDVIDLYQVHEWDGMTPIEETMEALDTLVRQGKVRYIGCSNYSGWHIMKALAAADKNHGQRFISQQIHYTLHSREAEYELVPISQDQGLGILIWSPLAGGLLSGKYRRDGGPESGRHVGGSREPPVPDWGKLYDIVEVIVAIAEARGVSGAQVALAWALGRPGVTSVIIGGRSEAQFKDNLAAADLKLTPEERQKLDAVSQPPLLYPYWHQSFTAQDRLSRIDLDLIGPYAEEFKRG

SEQ ID NO: 3 - protein, 353 aa, Artificial Sequence
  Enzyme
MDYRYLGRSGLRVSTLTMGTMTFGGSEKVGHTPQAEATRQIDLCLDHGINLLDTANVYNAGVSEEMIGVALAENGRRQKALIATKVRFRMGDGPNEVGLSRHHIIAQAEASLKRLKTDVIDLYQVHEWDGMTPIEETMEALDTLVKQGKVRYIGCSNYSGWHIMKALAAADKSHGQRFISQQIHYTLHSREAEYELVPISQDQGLGILIWSPLAGGLLSGKYRRDGGPESGRHVGGSREPPVPDWDKLYDIVDVIVAIAEERGVSGAQVALAWALGRPGVTSVIIGGRSEAQFKDNLAAADLKLSDEERQKLDAVSRPPLLYPYWHQTFTANDRLGPADQDLLSTYVEDFKRG

SEQ ID NO: 4 - protein, 353 aa, Artificial Sequence
  Enzyme
MEYRYLGRSGLKVSTLTMGTMTFGGSEKVGATAQDDATRQIDLCLDAGINLLDTANVYNAGVSEEMIGVALAENGRRQKALVATKVRFKMGDGPNEIGLSRHHIIAQAEASLKRLKTDVIDLYQVHEWDGMTPIEETMEALDTLIKQGKVRYIGCSNYSGWHIMKALQAADKNHGQRFISQQIHYTLHSREAEYELIPITGDQGLGVLIWSPLAGGLLSGKYRRNGGPDSGRHVGGFREPPVYDWEKLYDIVDVIVDIADDRGVSGAQVALAWSLGRPGVTSVIIGGRNDAQFKDNLAAAELKLTAEERARLDAVSRPPLLYPYWHQTFTAQDRLGPVDRNLIEPYAEELNRG

SEQ ID NO: 5 - protein, 353 aa, Artificial Sequence
  Enzyme
MQYRYLGRSGLKVSTLTMGTMTFGGGEKIGGTGQDEANRQIDLCLDHGINLLDTANVYNAGVSEEMIGVALSENGRRQKALIATKVRFKMGEGPNEVGLSRHHIIAQAEASLKRLKTDVIDLYQVHEWDGMTPIEETMEALDTLVKQGKVRYIGCSNYSGWHIMKALAAADSRHQQRFVSQQIHYTLHSREAEYELVPITQDQGLGILVWSPLAGGLLSGKYRRDGGPDAGRHVGGFREPPVPDWNRLYDIVDALVAIAEARGVSGAQVALAWLLGRPGVTSVIIGGRSEAQFRDNLAAADLQLTADERQRLDAVSQPPLLYPYWHQTFTANDRLGPADRDLLTPYVEEFKRG

SEQ ID NO: 6 - protein, 353 aa, Artificial Sequence
  Enzyme
MDYRYLGRSGLKVSAMTMGTMTFGGSERVGHTDLAGAARQVDLCLDAGINLYDSANVYNAGVSEDILGQVLAENGRRQRALVATKVRFKMGNGPNEAGLSRHHIIAQAEASLKRLRTDAIDLYQVHEWDGMTPIEETMEALDTLVRQGKVRYVGCSNYSGWHIMKALMAADKRQGQRFVSQQIHYSLHSRDAEYELVPISQDQGLGILVWSPLAGGLLSGKYRRTGGPESGRHVGGFREPPVYDWDKLYDLIDVIVDIAAQRGVSGAQVALSWLLERPGVTSLIIGGRNEAQFADNIAAIHLKLSSEERARLDAASRPPLLYPYWHQSFTAQDRLSRIDLDLIEPYAEEFKRG

SEQ ID NO: 7 - protein, 353 aa, Artificial Sequence
  Enzyme
MEYRYLGRSGLRVSVLTMGTMTFGGSEKIGNTSPADAARQVDMCLDAGINLYDTANVYNAGVSEEILGAILAENGRRQKALIATKVRFKMGDGPNEAGLSRHHIIEQCKASLKRLKTDVIDLYQVHEWDGRTPIEETMEALDTLVRHGHVRYIGCSNYSGWHIMKALASADQRHNARFVSQQIHYSLHSREAEYELVPISQDQGLGILVWSPLAGGLLSGKYRRSGGPETGRHVGGFREPPVYDQEKLYDVIEEIVAIAEDRGVSGAQVALAWLLGRPGVTSLIIGGRNEKQFADNIAAADFKLSAEERARLDKVSRPPLLYPYWHQSFSSQDRLSPVDMDLIGPYAEEFKRG

SEQ ID NO: 8 - protein, 353 aa, Artificial Sequence
  Enzyme
MDYRYLGRSGLKVSSMTMGTMTFGGSEKIGNTSRQDAARQVDMCLDAGINLYDSANVYNAGVSEEILGDILAENGRRQKALIATKVRFKMGDGPNEAGLSRHHIIEQCKASLKRLKTDVIDLYQVHEWDGQTPIEETMEALDILVRHGHVRYIGCSNYSGWHISKALAAADQRHNARFVSQQIHYSLHSRDAEYELVPISQDQGLGILVWSPLAGGLLSGKYRRDSAPDSGRHVGGFREPPVYDWDKLYSVIDVLVAVAEERGVSGAQVALSWLMGRPGVTSVIIGGRNEKQFADNIAAAQLVLSDEERARLDAASRPPLLYPYWHQSFTAQDRLGKIDMDLIGPYAEEFKRG

SEQ ID NO: 9 - protein, 350 aa, Artificial Sequence
  Enzyme
MEYRLLGRSGLKVSTLTMGTMTFGGNPKVGNTSLKDAQRQIDMCLEAGINMLDTANVYTRGVSESIIGEALTDGRRQRTLLATKVRFPMDDTDPNERGLSRYHIVNQCEASLKRLKTDVIDLYQVHEWDGQTPLEETMEALDMLVRHGKVRYIGCSNYSGWHIMKALGVSEKDARQRFVSQQIHYTLFSREAENELVPISLDQGLGILIWSPLAGGLLSGKYRRGQTAPEGARHAGGFKEPPVHDWERLYDIVEVLVSIAEVRGVSGAQIALAWLLGRPGVTSVIIGGRTEDQFRDNLAAAELKLTEHERKRLDDVSLLPLQYPYWHQSFTASDRLGPADLALHAPHLEK

SEQ ID NO: 10 - protein, 353 aa, Artificial Sequence
  Enzyme
MDYRYLGRSGLKVSVLSVGTVTFGGDGLWGDTDVTGAARQIDMCLDAGINLIDTANVYNKGVSEEITGEVLRDGGRRQRALIATKVRFPFGDGPNDRGLSRHHIIAQCEGSLKRLQTDVIDLYQVHQWDGQTPLEETMEALDTLVRQGKVRYIGCSNYSGWHLMKALAVADSRGYQRFVAQQIHYTLYSREAEYELQPITVDQGLGILVWSPLAGGWLSGKYTRASQPEDGRHVRGFREPPVPDPERLYDIVDVINAVAAERGVSGAVVSLAWALQRKGVSSVIVGARTDAQFADNLKAADLKLSDDEVARLDAVSQRPLPYPYWHQSFTAQDRLSEADLVLLAPYLEEYKRG

SEQ ID NO: 11 - protein, 348 aa, Artificial Sequence
  Enzyme
MDYRLLGRSGLKVSSLSIGTATFGGDGLWGDTNVKEAQRQIDLCLDHGVNLIDTANVYSGSVSETIIGEALTDGRRDRLLIATKVRFPRGKGPNDRGLSRWHIIREAEASLKRMKTDVIDLYQVHEWDGQTPLEETLEALDTLVRSGKVRYIGCSNYSAWHLMKALAVSNERNYQRFVSQQIHYTLHSREAEFELIPAGLDQGVSVLVWSPLAGGWLSGKYTRDSKPSDGRQVRGFKEPPIYDPEHLWKIVDVVNDVAGARGVSGAQVSLAWLLSKPIVASVIVGGRNIGQFEDNLKAAELTLTTEELQKLDAVSQPNLPYPYWHQSFTAQDRLGEPDLALHRPYLDK

SEQ ID NO: 12 - protein, 348 aa, Artificial Sequence
  Enzyme
MDYRLLGRSGLKVSSLSIGTATFGGDGLWGDTNVKEAQRQIDLCLDHGVNLIDTANVYSGSVSETIIGEALTDGRRDRLLIATKVRFPRGKGPNDRGLSRWHIIREAEASLKRMKTDVIDLYQVHEWDGQTPLEETLEALDTLVRSGKVRYIGCSNYSAWHLMKALATSNERNYQRFVSQQIHYTLHSREAEFELIPAGLDQGVSVLVWSPLAGGWLSGKYTRNSKPSDGRQVRGFKEPPIYDPEHLWKIVDVVNEVASAHGVSGAQVSLAWLLSKPIVASVIVGGRNIEQFEDNLKAAELQLTAEELGRLDAVSQPNLPYPYWHQNFTAQDRLSEPDLALHRPYLDK

SEQ ID NO: 13 - protein, 351 aa, Artificial Sequence
  Enzyme
MEYRLLGRSGLKVSTLTMGTMTFGGQGKFASVGNSGVDEARRLIDMCIDAGVNLIDTANVYSDGRSEEIIGEVLGGKRPKDVLIATKARFPMGDGPNNGGLSRYHLIRECEASLKRLRTDVIDLYQVHQWDGLTPLEETLEALDTLVRDGKVRYLGCSNYSAWHLMKALGISEREHRQRFVSQQIHYTLEAREAEYELLPISIDQGLGVLVWSPLAGGLLSGKHRRDGKAPEGSRQLEGWTEPPIRDEERLWRIVDVLVAIAEARGVSGAQVALAWLLERPAVTSLVIGGRTEAQFKDNLAAAELKLTAEERQRLDEVSAPPVLYPYWHQLMTASDRLGPADMPLLAPHLK

SEQ ID NO: 14 - protein, 351 aa, Artificial Sequence
  Enzyme
MEYRLLGRSGLKVSTLTMGTMTFGGQGKFASVGSSGVDEARRLIDMCIDAGVNLIDTANVYSDGRSEEIIGEVLGGKRPKDVLIATKARFPMGDGPNHGGLSRYHLIRECEASLKRLRTDVIDLYQVHQWDGLTPLEETLEALDTLVRDGKVRYLGCSNYSAWHLMKALGVSEREHRQRFISQQIHYTLEAREAEYELLPISIDQGLGVLVWSPLAGGLLSGKHRRDTKAPEGSRQLAGWTEPPIRDEERLWRVVDVLVSIAQSRGVSGAQVALAWLLERPAVTSLVIGGRTEAQFKDNLAAAELKLTAEERQRLDEVSAPPVLYPYWHQLMTASDRLGPADMPLLAPHLK

SEQ ID NO: 15 - protein, 343 aa, Artificial Sequence
  Enzyme
MEYRKLGNSGTVVTSYCLGTMTFGQETDEATSHLIMDDYIKAGGNFIDTANVYSAGVSEEIVGRWLKARPSEARQVVVATKGRFPMGAGPNDLGLSRTNLNRALNDSLRRLGVEQIDLYQMHAWDAVTPIEETLRFLDDAVSAGKIAYYGFSNYLGWQVTKAVHVARANHWTAPVTLQPQYNLLVRDIEHEIVPACQDAAMGLLPWSPLGGGWLAGKYQRDVMPSGATRLGENPNRGMESYGPRNAQERTWQIIDMVAEIAKERGVSAAQVALAWVVARPAVTAVILGARTREQLADNLGAVAVTLSTEEMERLNRVSAPAMADYPYGERGVSQRHRKMDGGR

SEQ ID NO: 16 - protein, 342 aa, Artificial Sequence
  Enzyme
MDYRKLGPSGTVVTAYCLGTMTGAEADEAASHKLLDDYFAWGGNFIDTADVYSAGKSEEIIGRWLKARPTEARQAIVATKGRFPMGNGPNDIGLSRRHLSQALDDSLRRLGLEQIDLYQMHAWDALTPIEETLRFLDDAVSSGKIGYYGFSNYVGWHIAKASEIAKARGYTRPVTLQPQYNLLMRDIELEIVAACQDAGMGLLPWSPLGGGWLTGKYKRDEMPTGATRLGENPNRGGESYAPRNAQERTWAIIGTVEEIAKARGVSMAQVALAWTAARPAITSVILGARTPEQLADNLGAMKVELSGEEMARLNEVSAPQPLDYPYGKGGINQRHRKIEGGR

SEQ ID NO: 17 - protein, 9 aa, Artificial Sequence
  motif
  MISC_FEATURE (1)..(1): X is not M or X is V, I, L, M, F or A.
  MISC_FEATURE (3)..(3): X is not A or X is E, D, Q or N.
  MISC_FEATURE (6)..(6): X is not A or X is G or A.
  MISC_FEATURE (7)..(7): X is not V or X is M, L, F, I, R, K, Q, N, E, V, A, or Norleucin.
  MISC_FEATURE (7)..(7): X is not V and/or X is M, L, F, I, R, K, Q, N, E, V, A, or Norleucin.
XHXWDXXTP

SEQ ID NO: 18 - skipped

SEQ ID NO: 19 - protein, 10 aa, Artificial Sequence
  motif
  MISC_FEATURE (1)..(1): X is G, R, K, Q, N, A, V, L, I, S, T, E, D
  MISC_FEATURE (3)..(3): X is not M or G or X is W, S, T, F, L, V, I, A or Y
  MISC_FEATURE (4)..(4): X is not E or X is T, S, R, Q, N or K.
  MISC_FEATURE (4)..(4): X is not E and/or X is T, S, R, Q, N or K.
  MISC_FEATURE (5)..(5): X is not S and/or X is E, D or Q.
  MISC_FEATURE (5)..(5): X is not S and/or X is E, D or Q.
  MISC_FEATURE (5)..(5): X is not S and/or X is P or A.
  misc_feature (6)..(7): Xaa can be any naturally occurring amino acid
  MISC_FEATURE (8)..(8): X is not P and/or X is I, L, M, A, F or V.
  MISC_FEATURE (9)..(9): X is R, K, Q, N, P, A, Y, W, F, T, S, H.
  MISC_FEATURE (10)..(10): X is not N and/or X is D, E or N.
XGXXXXXXXX

SEQ ID NO: 20 - protein, 9 aa, Artificial Sequence
  motif
VHEWDGMTP

SEQ ID NO: 21 - protein, 9 aa, Artificial Sequence
  motif
VHEWDGRTP

SEQ ID NO: 22 - protein, 9 aa, Artificial Sequence
  motif
VHEWDGQTP

SEQ ID NO: 23 - protein, 9 aa, Artificial Sequence
  motif
VHQWDGLTP

SEQ ID NO: 24 - protein, 9 aa, Artificial Sequence
  motif
VHQWDGQTP

SEQ ID NO: 25 - protein, 10 aa, Artificial Sequence
  motif
GGFREPPVYD

SEQ ID NO: 26 - protein, 10 aa, Artificial Sequence
  motif
GGSREPPVPD

SEQ ID NO: 27 - protein, 10 aa, Artificial Sequence
  motif
GGFREPPVPD

SEQ ID NO: 28 - protein, 10 aa, Artificial Sequence
  motif
GGFKEPPVHD

SEQ ID NO: 29 - protein, 10 aa, Artificial Sequence
  motif
RGFREPPVPD

SEQ ID NO: 30 - protein, 10 aa, Artificial Sequence
  motif
EGWTEPPIRD

SEQ ID NO: 31 - protein, 10 aa, Artificial Sequence
  motif
AGWTEPPIRD

SEQ ID NO: 32 - protein, 10 aa, Artificial Sequence
  motif
RGFKEPPIYD

SEQ ID NO: 33 - protein, 34 aa, Artificial Sequence
  motif
SPLAGGLLSGKYRRDGGPDAGRHVGGFREPPVYD

SEQ ID NO: 34 - protein, 34 aa, Artificial Sequence
  motif
SPLAGGLLSGKYRRDGGPESGRHVGGSREPPVPD

SEQ ID NO: 35 - protein, 34 aa, Artificial Sequence; identical to SEQ ID NO: 34
  motif

SEQ ID NO: 36 - protein, 34 aa, Artificial Sequence
  motif
SPLAGGLLSGKYRRNGGPDSGRHVGGFREPPVYD

SEQ ID NO: 37 - protein, 34 aa, Artificial Sequence
  motif
SPLAGGLLSGKYRRDGGPDAGRHVGGFREPPVPD

SEQ ID NO: 38 - protein, 34 aa, Artificial Sequence
  motif
SPLAGGLLSGKYRRTGGPESGRHVGGFREPPVYD

SEQ ID NO: 39 - protein, 34 aa, Artificial Sequence
  motif
SPLAGGLLSGKYRRSGGPETGRHVGGFREPPVYD

SEQ ID NO: 40 - protein, 34 aa, Artificial Sequence
  motif
SPLAGGLLSGKYRRDSAPDSGRHVGGFREPPVYD

SEQ ID NO: 41 - protein, 35 aa, Artificial Sequence
  motif
SPLAGGLLSGKYRRGQTAPEGARHAGGFKEPPVHD

SEQ ID NO: 42 - protein, 34 aa, Artificial Sequence
  motif
SPLAGGWLSGKYTRASQPEDGRHVRGFREPPVPD

SEQ ID NO: 43 - protein, 34 aa, Artificial Sequence
  motif
SPLAGGWLSGKYTRDSKPSDGRQVRGFKEPPIYD

SEQ ID NO: 44 - protein, 34 aa, Artificial Sequence
  motif
SPLAGGWLSGKYTRNSKPSDGRQVRGFKEPPIYD

SEQ ID NO: 45 - protein, 35 aa, Artificial Sequence
  motif
SPLAGGLLSGKHRRDGKAPEGSRQLEGWTEPPIRD

SEQ ID NO: 46 - protein, 35 aa, Artificial Sequence
  motif
SPLAGGLLSGKHRRDTKAPEGSRQLAGWTEPPIRD

SEQ ID NO: 47 - DNA, 771 bp, Artificial Sequence
  enzyme
atgacccgatttgcccattatcccagcctgaccgatatgcccgtcgtcatctcaggcggtgcctcgggcatcggcgaaagcctggtgcgaaactttgccgcccagggcgccagggtcggtttcgtcgatatcgccgtcgacgccggtgaacgcctcgccgccgaattgacggggcaggggcaaagcgtagccttcaccgcctgcgacatcaccgatacccaggcctatcaatccgccattgccggcttcgccgccacccatggcgatgccctggccctggtcaacaatgccgcccatgaccagcgccacgattgggctgaggtcacccctgcctattgggacgatcgcatggcggtcaacctcaagcatgcctttttcgccatccaggccgtggcgccgggcatggtccgcgccgggcgcggctccatcatcaataccggctcgatcagctggatgatcatgtcctcccgcattcccgtctatgaaaccgccaaggccgccatccatggcctcacccgcggcatggcgcgcgaactggggcagtcgggcattcgcgtcaattccctggtgcccggctgggtcatgaccgagcggcaattgacccattggctcgatgccgagggcgagcgggccatcgcacaaaaccaggtgctggccggccgggtctatcccgacgatgtcgcgcgcatggccctgttccttgccgccgacgacagcgccatgatttcggcccagcaatttgtcgtcgatggcggctgggccaatgcctga

SEQ ID NO: 48 - DNA, 1086 bp, Artificial Sequence
  enzyme
atgagccgcattttcaacgtcgccatcgtcggggtcggcatcggccgcagccacctggtcgagggctatgtgcccaatgccgacaaatacaaggtcgtcgcgctgtgcgatctcaatgtcgagcgcatgacgcccattgccgacgaattcggcgtcgagcgccgcatcaccaatttcgacgatatcctcgccatggacgatatcgacatcatcgatatctgcaccccgccgggcctgcattatcccatggtcatggcggcgctgaaggccggcaagcatgtaatctgcgaaaagccgctggtcggctcgctcgcccaggtcgatgaagtcattgcccaggaaaagatctccaagggcaagctgatgccggtgttccagtatcgctttggcgacggcatcgaacaggccaaggccatcatcgatgccggcattgccggcaagccattcgtcggcacggtggaaaccatgtggcgccgtggccccgattattatgccgtgccatggcgcggcaaatgggccaccgaactgggcggcgtgctgatgacccatgccatccaccagcacgatctcttcacctatctcatgggcgatgtgacgcggctcttcggccgggtcgccacccgcgtcaacgccattgaagtggaagactgcgttaccgccagccttgagctcgaaaatggcgccctgggcagctttaccgccacgctgggcgcagccgaggaaatcacaaggctgttcctgaccttcgagaacgtcaccttcgaaagcgattacgaggcctataatcccggcgccaagccgtggcgcatccagccgcgcaatcccgagacggcggcgaaaatcgacgccctgctcaaggactggaagcatgtgccctcgcgtttcgaaacgcagatggcccgcttccatgcggccctcttgggtgaagcgccgatgccggtgacctcggccgattcgcgccgggcgctggaaatcgtcaccgccttctaccattcctcgactacccacgaagatgtggccctgcccatcgcgtccgaccatccgcgttatcagagctgggttccgccccagttccgcgctgcctga

SEQ ID NO: 49 - DNA, 1062 bp, Artificial Sequence
  enzyme
atggactatcgctatctcggccgctcgggccttagggtttcggtgctgaccatgggcacaatgacctttggcggctcggaaaaggtggggcatacagcccaggccgatgcgacgcgccagattgatctctgccttgatcacggcatcaacctgctcgacaccgccaatgtctataatgccggggtctccgaggagatgatcggggtggcgctgagcgaacatggccggcggcaaaaggctttgattgccaccaaggtgcgcttcaggatgggtaacgggcccaatgaagtggggctgagccggcatcatatcattgcccaggccgaggcgagcctcaagcggctcaagaccgatgtcatcgatctctaccaggtgcatgaatgggatgggatgacgcccatcgaggagacgatggaagcgctcgatacgctcgtgaaacagggcaaggtgcgctatgtcggctgctcgaattattcgggctggcacatcatgaaggcgctggctgcggccgacaaacatcatggccagcgcttcatctcccagcagatccactacacgctgcattcgcgcgaagccgaatatgaactggtgccgatcagccaggaccaggggctgggtattctgatttggtcgccgctggcgggcggactgctctcgggcaagtatcgtcgcgatggcgggcccgatgccggccgccatgttggaggcttccgcgagccgccggtttatgactgggacaagctctacgacattatcgacgtcatcgtcgccattgcccgggagcgcgatgtgtcgggcgcgcaggtggcgttggcctgggcattggggcggccgggcgtgacctcggccattatcggtggccgtagcgaggcccagttccgcgacaatctggcggcggccgaactcaagctgaccgatgacgagcgcgcccggctcgatgcggccagccggccgccattgctttatccctattggcaccagtcttttaccgcccaggaccggctggaccagatcgacctggacctgatcgggccctatgccgaggagtttaaacgtggctga

SEQ ID NO: 50 - DNA, 786 bp, Artificial Sequence
  enzyme
atggacttgaatttgcgcgacaaggttgccgtcattaccgggggaacggtggggatcggcctggccattgccgaaggcctggcggcggagggcgtcaatctggtgctggtggggcgcgacaagctgcgggctgacgatgcggcagcgcttgtggccgacaagttcgggattatcgccacggcgatcagcgcggatgtcgcgactgccgaagggtgcgatgccgtgatcaagggcacggccaaggcctttggtggcgccgatatcctgatcaacaatgccgggaccgggtcgaacgagaccattgccgaggccgatgatgccaaatggcaatattattgggacctgcatgtgatggcggccgtgcggctggcgcgggggctggtgccgggaatgaaaaagcggggcggcggcgtcgtgctgcacaatgcctcgatctgcgcggtgcagccgctctggtatgagccgatctacaacaccaccaaggccgccttgatgatgttttccaagacgctggccaatgaggtggtgggcgacaatattcgcgtcaataccatcaatcccgggctggtgctgacgcccgattgggtcaagaccgccaagcagattgccggcgaagatggctggcaggcgcatctgcaaggggtggccgacgaggcgggcggcatgaagcgcttcgcgacgcccgaggaattggccaatttcttcgtcttcatgtgttcggacagagccagctattccaccggctcgacctattttgtcgatggcggctggctcaagacggtttga

SEQ ID NO: 51 - DNA, 1038 bp, Artificial Sequence
  enzyme
atggaactcggactctattccttcgccgaaaacacgcccgatcccctgaacggccgccgcctgcaaagcccggccgaacgtctcaaggacctgctggaagaaatcgaactggccgaccagctcggcctatccttttacggcctgggcgaacaccaccgccccgactacaccgcttccgcgcccgtcaccatcctggccgccgccgccgcgcgcaccaagtcgatccgcctctctaccgcggtcaccgtgctcagctcggaagaccccatccgcgtctatcagcaattcgccacgctcgataatctcagcaatggccgcgccgagatcatggccggccgcggctccttcatcgagagcttccccctcttcgggctcgacctcaacgattacgacgcgctgttcgaggaaaagctcgaaatgctgctcaaaatccgcgaaggcggcaaggtcacctggcccggcagcacccataccaagcccatccccggcattgccatctatcccatcccggtccagcagcccctgccgctctggatcgccgtcggcggcacgccaaattccgttgcccgcgcggcctattacggcctgcccctgatgatcgccatcatcggcggtcagccgcgccagtttgcgccgctggtcgatttctaccgcgaaaccgctgaaaaggtcggccgcgaccccaaatcgctgcccgtcggcatcagctcgcacggcttcatcgccgccgacagccaggacgcccgcgacatcgccttccccgcccatagcgaggccatgagccgcatcggcaaggaacgcggttggccgcccaccacccgcgcccaattcgacgccggcgccacgcccaacggcgcctatttcatggggtctccgcaggaagtcatcgacaagattctgatgcagcacgaatggttcaaacacgaccgcttcggcctgcaattcagcgtcggcaccctgccccacgacaaggtcatgaaagccatcgagctttacggcaccgtggtcaagccggcggtggacaaggcgctaggctaa

SEQ ID NO: 52 - DNA, 1026 bp, Artificial Sequence
  enzyme
atgagcactgaaatcgtcaccgatgtcgttgtgattggcgcgggcccctgcgggctgtttgcggccttcgaactcgggctgctcgacctcaaatgccatttcatcgacattctggaccgccccggcgggcagtgcgccgagctttatcccgaaaagccgatctacgatattcccggcttcccggtggtgaccggccaggatctgaccgacaatctgatggcccagatcgcgcccttcgcccccgaattccacttcaaccgcatggtcaattcgatcgagaagcaggaagacggctcgtttaagctcgaaaccgacgccgacgagattttccacgcgaaggtcgtggtgatcgcggccggcggcggctcgttccagcccaagcgcccgccggtcgacaatatcgaagcctatgaaaacaagtcggttttctattcggtccgcaagatggacgatttccgtgaccaggacgtggtgatcgtcggcggcggcgattccgccctcgactggacgctcaacctgcagcccatcgtgcgctcgctgaccctggtacaccgccgcgatgccttcaaggccgcgcccgcttcggtcaacaagatgaaggaaatggtcgccgagggtaagatcaatttcctgctcggccaggtggccaagctcgatggcgaaaacggccagatcaaccacgtgcatctgaccaccgatgccggcgatctctcggtgcccgccacccgcctgctgcccttcttcggcctcaccatgaagctgggtccggtggccgattggggccttgagctcaatgacaatacgatcaaggtcgataccgaaaagttcgagacctcggtgcccggcattttcgccattggcgacatcaactggtatccgggcaagctcaagctgatcctctccggcttccacgaggctgccctcatggcccaggccgccaagaagattgtgtcgcccgacgagcgcgtggtgttccaatacaccaccagctccaccaagctgcagaagaagctgggcgtcgcctag

SEQ ID NO: 53 - DNA, 1062 bp, Artificial Sequence
  enzyme
atggactatcgctatctcgggcgctcgggcctgaaagtctcgagcatgaccatgggcaccatgacctttggcggcagcgaaaagatcggcaataccagccgacaggacgcggcgcggcaggtggatatgtgtctcgatgcgggcatcaacctctatgacagcgccaatgtctataatgcgggggtgtccgaggaaatcctgggcgacattctcgccgaaaacgggcggcggcagaaagcgctgatcgccaccaaggtacgcttcaagatgggcgatggccccaacgaggccgggctcagccgacaccatatcatcgagcagtgcaaggcgagcctcaaacgcctcaagaccgatgtgatcgacctctatcaggtgcatgaatgggatgggcagacccccatcgaggaaacgatggaagcgctcgacattctcgtgcgccacggccatgtgcgctatatcgggtgctccaattattcgggctggcatatttccaaggcccttgccgccgccgaccagcggcacaatgcgcgctttgtgtcccagcagatccattattcgctgcatagccgcgacgccgaatatgagctggtgccgatttcccaggaccaggggctgggcattctcgtctggtcgccgctggcgggcgggttgctttcgggcaagtatcgccgggacagcgcgccggacagcgggcggcatgtcggcgggttccgcgagccgccggtctatgactgggacaagctctattcggtcatcgacgtgctggtggcggtggccgaggagcgtggcgtttcgggggcgcaggtggcgctgagctggctgatgggacgcccgggcgtcacttccgtcatcatcggcggacgtaacgaaaagcagtttgccgacaatatcgcagcggcccagctcgtgctcagtgacgaggaacgcgcccggctcgatgcggccagccgaccgccgttgctctatccctactggcaccagtccttcaccgcgcaggatcggctgggcaagatcgacatggatttgatcggtccttatgccgaggagttcaagcgtggctga

SEQ ID NO: 54 - DNA, 1053 bp, Artificial Sequence
  enzyme
atggaataccgcttgctcgggcgctcgggactgaaggtctcgacccttaccatgggcacgatgacgttcggggggaacccgaaggtcggcaataccagcctcaaggacgcgcagcgccagatcgacatgtgtctggaggcgggcatcaacatgctcgacacggccaatgtctatacgcggggcgtgtcggaaagcattatcggggaggcactgaccgatgggcggcgccagcggacgctgctggcgaccaaggtgcgcttcccgatggacgacaccgaccccaacgagcggggactgtcgcgctaccacatcgtcaaccagtgcgaggcaagcctcaagcggctcaagaccgatgtgatcgacctctaccaggtgcatgaatgggacgggcagaccccgctcgaggagaccatggaagcgctcgacatgctcgtgcgccacggcaaggtccgctatatcggctgctcgaactattcgggctggcacatcatgaaggcgctcggcgtttccgagaaggacgcccggcagcgcttcgtctcccagcagatccactacacgctgttttcgcgcgaggcggagaacgagctggtgccgatcagcctcgaccaggggctgggcattctcatctggagcccgctggcgggcggcctgctttcgggcaagtatcgccgcggccagacggcgccggaaggggcgcgccatgccgggggcttcaaggagccgccggtgcatgactgggagcggctctacgatatcgtggaagtgctggtttcgatcgccgaggtgcgcggggtttcgggcgcgcagatcgcgctggcctggctgctggggcgcccgggggtgacctcggtgatcatcggcgggcgcacggaagaccagttcagggataacctggcggcggccgaactcaagctgaccgagcatgagcgcaagcggctagacgacgtgtcgctgctgccgctgcaatatccctactggcaccagagctttacggcctcggaccggctggggccggcggacctggcgctgcatgcaccccatctcgaaaaatag

SEQ ID NO: 55 - DNA, 1062 bp, Artificial Sequence
  enzyme
atggactaccgctatctcggccggtcgggcctcaaggtttcggtgctgagcgtcgggacggtgacgttcggcggcgacgggctgtggggcgatacggacgtcaccggcgccgcccggcagatcgacatgtgcctcgatgcaggcatcaacctcatcgataccgccaatgtctacaacaagggcgtttcggaagagatcaccggcgaggtgctgcgcgacggcggtcggcggcagcgcgcgctgatcgccaccaaggtgcgctttccgttcggcgacggtcccaatgaccgcgggctgtcgcgccaccacatcatcgcccagtgcgagggcagcctcaaacgcctccagaccgacgtcatcgatctctaccaggtccatcagtgggacgggcagacgcccctcgaggagacgatggaagccctcgataccctggtgcggcaggggaaggtccgctacatcggctgctcgaactattcgggctggcacctgatgaaggcgctcgccgtcgccgacagccgcggctaccagcggttcgtcgcccagcagatccactacaccctctattcgcgcgaggccgaatacgagctgcagccgatcaccgtcgaccaggggctcggcatactcgtctggagcccgctcgccggcgggtggctctcgggcaagtacacgcgcgccagccagcccgaggacggccgacacgtgcgcggtttccgcgagccgccggtgcccgatcccgagcggctctacgacatcgtcgatgtcatcaatgcggttgccgccgagcggggcgtttcgggcgcggtcgtttcgctggcttgggctttgcagcgcaagggcgtctcgtcggtgatcgtgggcgcgcgcaccgacgcgcagttcgccgataacctcaaggccgccgatctaaagctcagcgacgacgaggtcgcccggctcgacgccgtcagccagcgtccgcttccctatccctattggcaccagtccttcaccgcccaggaccgcttgagcgaagccgatctcgtgctgctcgccccttatctcgaggagtacaagcgtggctga

SEQ ID NO: 56 - DNA, 1047 bp, Artificial Sequence
  enzyme
atggactatcgattgctcggccgttccggcctcaaggtgtcgtcgctgtcgatcggcacggcgacgttcggcggcgacgggttgtggggcgacaccaacgtcaaggaggcgcagcgccagatcgacctctgcctcgaccacggcgtcaacctgatcgacaccgccaatgtctattcgggcagcgtgtcggagacgatcatcggcgaggcgctgaccgatggccggcgcgaccgcttgctgatcgccaccaaggtgcgcttccccaggggcaagggaccgaacgatcgcgggctcagccgatggcacatcatccgtgaggcggaagcctcgctgaagcggatgaagaccgacgtcatcgacctgtaccaggtgcatgagtgggatgggcagacgccgctcgaggagacgctggaagcactcgacaccctcgtccgctccggcaaggtccgctatatcggctgctcgaactattcggcctggcacctgatgaaggcgctcgcggtttccaacgagcgcaactaccagcgcttcgtttcccagcagatccactacacgctgcactcgcgcgaagccgagttcgagctgatcccggccggcctcgaccagggtgtctcggtgctggtgtggtcgccgctcgccggcgggtggctctcgggcaagtacacccgcgattccaagccgagcgacggccggcaggtgcgcggcttcaaggagccgccgatctacgatcccgagcatctgtggaagatcgtcgacgtggtcaacgacgtggcgggcgcgcgtggcgtttccggcgcgcaggtgtcgcttgcctggttgctgtcgaagccgatcgtcgcttcggtgatcgtcggcggccgcaatatcggacagttcgaagacaacctcaaagccgcggaactgactctcaccaccgaggagctgcagaagctcgacgcggtcagccagccgaacctgccctacccgtactggcaccagagctttaccgcgcaggaccggctcggtgagcccgacctggcgctgcaccgcccctatctcgacaagtga

SEQ ID NO: 57 - DNA, 1047 bp, Artificial Sequence
  enzyme
atggactatcgattgctcggccgttccggcctcaaggtctcgtcgctgtcgatcggcacggcgacgttcggcggcgatgggttgtggggcgataccaacgtcaaggaggcgcagcgccagatcgacctctgcctcgaccatggcgtcaacctgatcgacaccgccaacgtctattcggggagcgtctcggaaacgatcatcggcgaggcgctgaccgacgggcggcgtgatcggctgctgatcgccaccaaggtgcgcttcccacgcggcaaggggcccaatgatcgcggcctcagccgctggcacatcatccgcgaggcggaagcgtcgctcaaacggatgaagaccgacgtcatcgacctctaccaggtgcatgagtgggacgggcagacgccgctcgaggaaacgctggaggcgctcgatacgctcgtccgctcgggcaaggtccgctatatcggctgctcgaactattcggcctggcacctgatgaaggcgctcgccacctcgaacgagcgcaactaccagcgcttcgtctcccagcagatccactacacgctgcattcgcgtgaggccgagttcgagctgatcccggccgggctcgaccagggcgtttcggtgctggtgtggtcgccgctggccggcgggtggctgtcgggcaagtacacccgcaactcgaagccgagcgatggccggcaggtgcgcggcttcaaggagccgccgatctatgatccggagcacctgtggaagatcgtcgatgtggtcaacgaagtggccagcgcgcatggcgtctccggcgcgcaggtgtcgctggcctggctgttgagtaagccgatcgttgcctcggtgatcgtcggcggccgcaatatcgagcagttcgaggacaacctgaaagccgccgagctgcagctcaccgccgaggaactgggcagactcgacgcggtcagccagccgaacctcccctacccctactggcaccagaactttaccgcgcaggatcgcctcagcgagcctgacctggcgctgcaccggccctatctcgacaaatga

SEQ ID NO: 58 - DNA, 1056 bp, Artificial Sequence
  enzyme
atggaatatcgactgcttggccgctccggcctcaaagtctccaccctcacgatgggcacgatgaccttcggcggccagggcaagttcgcctcggtcggcaactccggcgtcgacgaagcacgccggctgatcgacatgtgcatcgatgccggcgtcaatctcatcgatacggcgaacgtctactccgatggccgttcggaagaaatcatcggcgaagtgctcggcggcaagcgtccgaaggacgtactgatcgcgaccaaggcacgctttccgatgggcgacggccccaacaacggcggcctctctcgctatcacctgattcgcgagtgcgaagcgagcctgaagcgcctgcgcacggacgtgatcgatctctaccaggttcaccagtgggatggcctgaccccgctggaagaaaccctggaagcgctcgacaccctggttcgcgacggcaaggtgcgttacctgggctgctccaactattccgcgtggcacctgatgaaggcgctcggcatcagtgagcgcgagcatcgccagcggttcgtcagccaacagatccattacacgctggaggcgcgcgaggccgaatacgagctgctgccgatctcgatcgaccagggcctcggcgtcctcgtctggagtccgcttgccggtggcctgctttcgggcaagcaccgtcgcgatggcaaggcaccggagggctcacgtcagctggagggctggaccgagccgccgatccgcgacgaagagcgcctttggcgcatcgtcgacgtgctggtggccatcgccgaagcgcgcggcgtgtcgggtgcacaggtcgcgctggcctggctgctcgagcgtcccgcggtgacctccctggtcatcggcggtcgtaccgaggcgcagttcaaggacaacctcgccgccgccgagctgaagctcacggccgaagagcgtcagcggctggacgaggtcagtgcgccgccggtgctctacccgtactggcaccagctgatgacggcgtcggaccgcctgggtccggcggacatgccattgctggcgccgcatctgaagtaa

SEQ ID NO: 59 - DNA, 1056 bp, Artificial Sequence
  enzyme
atggaataccgactgcttggccgctccggcctcaaagtctccaccctcacgatgggcacgatgaccttcggcggccagggcaaattcgcctcggtcggtagctccggcgtcgacgaagcgcgccggctgatcgacatgtgcatcgacgccggcgtgaatctcatcgacacggcgaacgtctattccgacggtcgttcggaagagattatcggtgaagtgctcggcggcaagcgtccgaaggacgtcctgatcgcgaccaaggcgcgctttcccatgggtgatggcccgaaccatggtggcctgtcgcgctatcacctgattcgcgaatgcgaagccagcctgaagcggctgcgcacggacgtgatcgatctctaccaggttcaccagtgggatggcctgacgcctctggaggaaaccctggaagcgctcgacaccctcgttcgcgacggcaaggtgcgttacctgggttgctccaactattccgcctggcacctgatgaaggcgctcggcgtgagcgagcgtgagcaccgccagcgtttcatcagccagcagatccattacacgctggaagcgcgcgaagccgaatacgaactgctgccgatttcgatcgaccagggcctcggcgtgctggtgtggagtccgctcgccggcgggctgctttcgggcaagcaccgtcgcgataccaaggccccggaaggctcgcgccagctggccggctggaccgaaccgccgatccgcgacgaagagcgcctgtggcgcgtcgtcgacgtactggtttcaatcgcccaatcgcgtggcgtgtcgggagcgcaggtcgcgctggcctggttgctcgagcgtcctgcggtcacctcgctggtgatcggtggtcgtaccgaggcacagttcaaggacaacctggcggccgccgaactgaagctcacggccgaagagcgtcagcgtctggatgaagtcagcgcgccgccggtgctctatccgtactggcaccagttgatgaccgcatcggatcgcctgggtccggccgacatgcccctgctggcgccgcacctcaaataa

SEQ ID NO: 60 - DNA, 1062 bp, Artificial Sequence
  enzyme
atggaataccgctatctcggccgctcaggcttgaaggtgtcgacattgaccatgggcaccatgacctttggcggctcggaaaaggttggggcgacggcgcaagacgatgcgacgcgccagatcgacctgtgcctcgatgcagggatcaatctgctcgacacggccaatgtctacaatgccggggtctccgaggaaatgattggcgtggcgctggccgagaatggtcgccgccagaaagcactcgtagccaccaaggtccgcttcaagatgggcgatgggcccaacgagatcggcctcagccgtcaccatattattgcccaggccgaagccagccttaagcgcttgaaaacagacgttattgatctctatcaggtccacgaatgggacggcatgacgcccatcgaggagacgatggaagcgctcgataccctgatcaagcagggcaaagtccgctatatcggctgctcaaattattcgggctggcatatcatgaaggcgctgcaggccgccgacaaaaaccacggccagcgcttcatcagccagcagatccactacacgctgcattcgcgcgaagccgaatatgaactgatcccgatcactggggatcaaggccttggcgtcctcatctggtcgccgctggccggtggtttgctctcgggcaaataccgtcgcaacggtggccctgacagcgggcgccatgtcggcggcttccgcgagccgccggtttatgactgggagaagctctacgacatcgtcgatgtgatcgtggatattgctgatgaccgcggcgtgtcgggtgcacaggttgcgctggcatggtcgctggggcggccgggtgtaacctcggtgatcatcggtggccgcaatgatgcccagttcaaagacaatctggcggcagccgagttgaagctgacggcggaagagcgcgcgcgacttgacgcggtcagccgtccaccgctgctctatccttattggcatcagacgtttacggcgcaggaccggttaggccctgtcgatcgaaacctgatcgaaccctatgcagaggaattgaaccgtggctga

SEQ ID NO: 61 - protein, 608 aa, Artificial Sequence
  enzyme
MRFEYLRQNVVGLALSTALIASLSGPAFAQHDANAAAEPSKAGQSAIENFQPVTADDLAGKNPANWPILRGNYQGWGYSPLDQINKDNVGDLQLVWSRTMEPGSNEGAAIAYNGVIFLGNTNDVIQAIDGKTGSLIWEYRRKLPSASKFINSLGAAKRSIALFGDKVYFVSWDNFVVALDAKTGKLAWETNRGQGVEEGVANSSGPIVVDGVVIAGSTCQFSGFGCYVTGTDAESGEELWRNTFIPRPGEEGDDTWGGAPYENRWMTGAWGQITYDPELDLVYYGSTGAGPASEVQRGTEGGTLAGTNTRFAVKPKTGEVVWKHQTLPRDNWDSECTFEMMVVSTSVNPDAKADGMMSVGANVPRGETRKVLTGVPCKTGVAWQFDAKTGDYFWSKATVEQNSIASIDDTGLVTVNEDMILKEPGKTYNYCPTFLGGRDWPSAGYLPKSNLYVIPLSNACYDVMARTTEATPADVYNTDATLVLAPGKTNMGRVDAIDLATGETKWSYETRAALYDPVLTTGGDLVFVGGIDRDFRALDAESGKEVWSTRLPGAVSGYTTSYSIDGRQYVAVVSGGSLGGPTFGPTTPDVDSASGANGIYVFALPEKK

SEQ ID NO: 62 - protein, 586 aa, Artificial Sequence
  enzyme
MKKRTSILLASVAMLGMGSTAFAQVDINALPAVTDAILANPDAGDWPSYGRDITNYRFSPLDQVNKDNVGQLTLAWARALEPGNLQSAPLEFGGVLFTAAPGDVVQAMDAATGQLIWEYRRQLPDRATLNSLGENKRGIALYEDKIYVATWDNFIVALDAKTGQVAWESDRGGGADLISNTTGPIVANGVVVAGSTCQFSEFGCYVTGHDAATGEELWRNNFIPKKGEEGDDTWGDSTEDQRWMTGAWGQMTYDPELDLVYYGSTGAGPAAEFQRNTVGGTLFGSNTRFAVKPKTGEIVWRHQVLPRDNWDQECTYEMVPVDIDSAPAADMEGLLALGTAAPGKKRVLTGVPCKTGVMWQFDAQTGEFIYARDTVQQTLIESVDNTGLVTVNEAAIPTEVDVATPMCPTYLGGRDWSPTAFNPTSKVMFVPLTNMCADVTVLDQEPTGLDVYNTELTYKMPEGVTDAGRIDAINVETGKTLWSWTQQTPQYASITATAGGLIFTGGADRRFKAIDQETGELVWSVTLGSRATGHPISYEVDGRQYIAIPAGGPGYATDLITASGSTVDVVSGSNMLYVFALPEQKK

SEQ ID NO: 63 - protein, 353 aa, Artificial Sequence
  enzyme
MDYRYIGRSGLRVSVLTMGTMTFGGSDKVGHTAQADATRQIDLCLDHGINLLDTANVYNAGVSEEMIGVALSEHGRRQKALIATKVRFRMGNGPNEVGLSKHHIIAQAEASLKRLKTDVIELYQVHEWDGMTPIEETMEALDTLVKQGKVRYVACSNYSGWHIMKALAAADKHHGQRFISQQIHYTLHSREADYELVPISQDQGLGILIWSPLAGGLLSGKYRRDGGPDAGRHVGGFREPPVYDWDKLYEIIDVIVAIARERDVSGAQVALAWALGRPGVTSAIIGGRSEAQFRDNLAAAELRLTDDERARLDAASRPPLLYPYWHQSFTAQERLDQIDLDLIGPYAEEFKRG

SEQ ID NO: 64 - protein, 353 aa, Artificial Sequence
  enzyme
MDYKYLGRSGLRVSVLTMGTMTFAGSEKVGHTAQADATRQIDLCIDHGINLLDTANVYNAGVSEEMIGVALSEHGRRQKALIATKVRFRMGNGPNEVGLSRHHLIAQAEASIKRLKTDVIDLYQVHEWDGMTPIEETMEALDTLVKQGKVRYVGCSNYSGWHIMKGLAAADKHHGQRFISQQIHYTLHSREAEYELVPISQDQGLGILIWSPLAGGLLSGKYRRDGGPDAGRHVGGFRDPPVYDWDKLYEILDVIVAIAREKDVSGAQVALAWALGRPGVTSAIIGGRSEAQFRDNLAAAELRLTDDERARLDAASRPPLLYPYWHQSFTGQDRLDQVDLDLIGPYAEEFKRG

SEQ ID NO: 65 - protein, 353 aa, Artificial Sequence
  enzyme
MDYKYLGRSGIRVSVLTMGTMTFAGSEKVGHTAQADATRQIDLCLDHGINLLDTANVYNAGVSEEMIGVALSEHGRRQKALIATKVRFRMGNGPNEVGLSRHHLIAQAEASLKRIKTDVIDLYQVHEWDGMTPIEDTMEALDTLVKQAKVRYVGCSNYSGWHIMKALAGADKHHGQRFISQQIHYTLHSREAEYELVPISQDQGLGILIWSPLAGGLLSGKYRRDGGPDAGRHVGGFRDPPVYDWDRLYDIIDVIVAIAREKDVSGAQVALAYALGRPGVTSAIIGGRSEAQFRDNLGAAELKLTDDERARLDAASRPPLLYPYWHNSFTGQDRLDQVDLDLIGPYAEEFKRG

SEQ ID NO: 66 - protein, 353 aa, Artificial Sequence
  enzyme
MDYRFLGRSGIRVSVLTMGTMTFGGTEKVGHTAQADATRQLDICLDHGINLLDTANVYNAGVSEEMIGVALSEHGKRQKALIATKVRFRMANGPNEVGLSRHHIIAQAEASLKRIKTDVIDLYQVHEWDGMTPIDETLEALDTLVKQGKVRYVGCSNYSGWHIMKGLAAADKHHGQRFISQQIHYTLHSREGEYELVPISQDQGLAILIWSPLAGGLLSGKYKRDGGPDAGRHVGGFREPPLYDWDRLYDIIDVIVAIARERDVSGAQVALAFALGRPGVTSAIIGGRSEANFRDNLGAAELRLSDDERARLDAASRPPLLYPYWHQSFTANDRLDQLDLDLIGPYADEFKRG

SEQ ID NO: 67 - protein, 353 aa, Artificial Sequence
  enzyme
MDYKYIGRSGIRVSVLTMGTMTFAGSERVGHTGQAEATRQLDICLDHGINLLDTANVYNAGVSEEMLGVGLSEHGRRQKALIATKVRFRMANGPNEVGLSRHHIIAQAEASIKRLKTDVIELYQVHEWDGMTPIDETMEALDTLVKQAKVRYVACSNYSGWHIMKGLAGADKHHGQRFISQQIHYTLHSRDGEYELVPISQDQGLAILIWSPLAGGLLSGKYRRDGGPDAGRHVGGFREPPVYDWDKLYEILDVIVAIARERDVSGAQVALAWALGRPGVTSAIIGGRSEAQFRDNIGAADLKLSDEERARLDAASRPPLLYPYWHNSFTGNDRLDQLDLDLLGPYADEFKRG

SEQ ID NO: 68 - protein, 353 aa, Artificial Sequence
  enzyme
MDYKYLGRSGIRVSVLTMGTMTFAGSERVGHTGQAEATRQLDICLDHGINLLDTANVYNAGVSEEMLGVGLSEHGRRQKALIATKVRFRMANGPNEVGLSRHHIIAQAEASLKRLKTDVIELYQVHEWDGMTPIEDTMEALDTLVKQAKVRYVGCSNYSGWHIMKGLAGADKHHGQRFISQQIHYTLHSRDAEYELVPISQDQGLGILIWSPLAGGLLSGKYRRDGGPDAGRHVGGFREPPVYDWDKLYELIDVIVAIARERDVSGAQVALAWALGRPGVTSAIIGGRSEAQFRDNIAGAELKLSDDERARLDAASRPPLLYPYWHQSFTGNDRLDQIDLDLLGPYADEFKRG

SEQ ID NO: 69 - protein, 353 aa, Artificial Sequence
  enzyme
MDYKYIGRSGIRVSVLTMGTMTFGGSEKVGHTGQADATRQIDICLDHGINLLDTANVYNAGVSEEMLGVALSEHGRRQKALIATKVRFRMGNGPNEVGLSRHHIIAQAEASLKRLKTDVIELYQVHEWDGMTPIDETMEALDTLVKQAKVRYVACSNYSGWHIMKGLAAADKHHGQRFISQQIHYTLHSREGEYELVPISQDQGLAILIWSPLAGGLLSGKYRRDGGPDAGRHVGGFREPPVYDWDKLYDILDVIVAIARERDVSGAQVALAWALGRPGVTSAIIGGRSEAQFRDNIGAAELKLTDEERARLDAASRPPLLYPYWHNSFTGQDRLDQLDLDLLGPYADDFKRG

SEQ ID NO: 70 - protein, 353 aa, Artificial Sequence
  enzyme
MDYKYLGRSGLRVSVLTMGTMTFGGSERVGHTAQAEATRQIDLCLDHGINLLDTANVYNAGVSEEMLGVALSEHGRRQKALIATKVRFRMGNGPNEVGLSRHHIIAQAEASLKRLKTDVIELYQVHEWDGMTPIEDTMEALDTLVKQGKVRYVACSNYSGWHIMKGLAAADKHHGQRFISQQIHYTLHSREAEYELVPISQDQGLGILIWSPLAGGLLSGKYRRDGGPDAGRHVGGFREPPVYDWDKLYEILDVIVAIARERDVSGAQVALAWALGRPGVTSAIIGGRSEAQFRDNIGAADLKLSDEERARLDAASRPPLLYPYWHQSFTANDRLDQLDLDLIGPYAEDFKRG

SEQ ID NO: 71 - protein, 353 aa, Artificial Sequence
  enzyme
MDYRYLGRSGLRVSVLTMGTMTFAGSEKVGHTGQADATRQIDLCLDHGINLLDTANVYNAGVSEEMIGVGLSEHGRRQKALIATKVRFRMANGPNEVGLSRHHIIAQAEASIKRLKTDVIDLYQVHEWDGMTPIDETMEALDTLVKQGKVRYVACSNYSGWHIMKGLAGADKHHGQRFISQQIHYTLHSREGEYELVPISQDQGLAILIWSPLAGGLLSGKYRRDGGPDAGRHVGGFREPPVYDWDKLYDILDVIVAIARERDVSGAQVALAWALGRPGVTSAIIGGRSEAQFRDNIAAAELKLSDDERARLDAASRPPLLYPYWHQSFTGQDRLDQIDLDLLGPYAEEFKRG

SEQ ID NO: 72 - protein, 353 aa, Artificial Sequence
  enzyme
MDYRYIGRSGLRVSVLTMGTMTFGGSEKVGHTGQADATRQIDICLDHGINLLDTANVYNAGVSEEMLGVGLSEHGRRQKALIATKVRFRMANGPNEVGLSRHHIIAQAEASIKRLKTDVIDLYQVHEWDGMTPIEDTMEALDTLVKQGKVRYVACSNYSGWHIMKALAGADKHHGQRFISQQIHYTLHSREAEYELVPISQDQGLGILIWSPLAGGLLSGKYRRDGGPDAGRHVGGFREPPVYDWDKLYDLIDVIVAIARERDVSGAQVALAWALGRPGVTSAIIGGRSEAQFRDNIGAADLKLTDDERARLDAASRPPLLYPYWHNSFTANDRLDQIDLDLIGPYAEDFKRG

SEQ ID NO: 73 - protein, 353 aa, Artificial Sequence
  enzyme
MDYRYLGRSGLRVSVLTMGTMTFGGSEKVGHTGQADATRQLDLCLDHGINLLDTANVYNAGVSEEMIGVGLSEHGRRQKALIATKVRFRMGNGPNEVGLSRHHIIAQAEASLKRLKTDVIELYQVHEWDGMTPIEDTMEALDTLVKQAKVRYVACSNYSGWHIMKALAGADKHHGQRFISQQIHYTLHSREAEYELVPISQDQGLAILIWSPLAGGLLSGKYRRDGGPDAGRHVGGFREPPVYDWDKLYEIIDVIVAIARERDVSGAQVALAWALGRPGVTSAIIGGRSEAQFRDNLAAAELKLTDEERARLDAASRPPLLYPYWHQSFTAQDRLDQLDLDLIGPYAEDFKRG

SEQ ID NO: 74 - protein, 353 aa, Artificial Sequence
  enzyme
MDYRYIGRSGIRVSVLTMGTMTFGGSERVGHTAQADATRQLDLCLDHGINLLDTANVYNAGVSEEMIGVALSEHGRRQKALIATKVRFRMANGPNEVGLSRHHIIAQAEASIKRLKTDVIELYQVHEWDGMTPIEETMEALDTLVKQAKVRYVGCSNYSGWHIMKALAGADKHHGQRFISQQIHYTLHSREGEYELVPISQDQGLGILIWSPLAGGLLSGKYRRDGGPDAGRHVGGFREPPVYDWDKLYDLIDVIVAIARERDVSGAQVALAWALGRPGVTSAIIGGRSEAQFRDNLGAAELKLTDEERARLDAASRPPLLYPYWHQSFTGNDRLDQIDLDLLGPYADEFKRG

SEQ ID NO: 75 - protein, 353 aa, Artificial Sequence
  enzyme
MDYRYIGRSGIRVSVLTMGTMTFAGSERVGHTAQADATRQLDICLDHGINLLDTANVYNAGVSEEMLGVGLSEHGRRQKALIATKVRFRMANGPNEVGLSRHHIIAQAEASLKRLKTDVIELYQVHEWDGMTPIDETMEALDTLVKQAKVRYVACSNYSGWHIMKGLAGADKHHGQRFISQQIHYTLHSRDGEYELVPISQDQGLAILIWSPLAGGLLSGKYRRDGGPDAGRHVGGFREPPVYDWDKLYELIDVIVAIARERDVSGAQVALAWALGRPGVTSAIIGGRSEAQFRDNIGAADLKLSDDERARLDAASRPPLLYPYWHNSFTGNDRLDQLDLDLLGPYADEFKRG

SEQ ID NO: 76 - protein, 353 aa, Artificial Sequence
  enzyme
MDYRYLGRSGIRVSTLTMGTMTFAGSEKVGHTGQAEATRQLDICLDHGINLLDTANVYNAGVSEEMLGVGLSENGRRQKALIATKVRFRMANGPNEVGLSRHHIIAQAEASIKRLKTDVIELYQVHEWDGMTPIDETMEALDTLVKQAKVRYIACSNYSGWHIMKGLAGADKSHGQRFISQQIHYTLHSREAEYELVPISQDQGLAILIWSPLAGGLLSGKYRRDGGPDSGRHVGGSREPPVPDWDKLYEILDVIVAIAEERGVSGAQVALAWALGRPGVTSAIIGGRSEAQFRDNLGAADLKLSDEERQRLDAASRPPLLYPYWHNSFTGNDRLDPADLDLLGTYADEFKRG

SEQ ID NO: 77 - protein, 353 aa, Artificial Sequence
  enzyme
MDYRYLGRSGIRVSTLTMGTMTFAGSEKVGHTPQAEATRQLDLCLDHGINLLDTANVYNAGVSEEMIGVALAENGRRQKALIATKVRFRMGNGPNEVGLSRHHIIAQAEASLKRLKTDVIDLYQVHEWDGMTPIEDTMEALDTLVKQAKVRYIGCSNYSGWHIMKALAAADKSHGQRFISQQIHYTLHSREAEYELVPISQDQGLGILIWSPLAGGLLSGKYRRDGGPESGRHVGGSREPPVPDWDKLYDIIDVIVAIAEERGVSGAQVALAWALGRPGVTSVIIGGRSEAQFRDNLAAADLKLSDEERQRLDAASRPPLLYPYWHQTFTGNDRLGPADQDLLSTYVEDFKRG

SEQ ID NO: 78 - protein, 354 aa, Artificial Sequence
  enzyme
MDYRYLGRSGIRVSTLTMGTMTFGGSEKVGHTGQADATRQIDICLDHGINLLDTANVYNAGVSEEMLGVALSENGRRQKALIATKVRFRMGNGPNEVGLSRHHIIAQAEASLKRLKTDVIELYQVHEWDGMTPIDETMEALDTLVKQAKVRYIACSNYSGWHIMKGLAAADKSHGQRFISQQIHYTLHSREAEYELVPISQDQGLAILIWSPLAGGLLSGKYRRDGGPDSGRHVGGSREPPVPDWDKLYDILDVIVAIAEERGVSGAQVALAWALGRPGVTSAIIGGRSEAQFRDNLGAADLKLTDEERQRLDAASRPPLLYPYWHNSFTGQDRLGPADQDLLLSTYVEDFKRG

SEQ ID NO: 79 - protein, 353 aa, Artificial Sequence
  enzyme
MDYRYLGRSGLRVSTLTMGTMTFGGSEKVGHTAQAEATRQIDLCLDHGINLLDTANVYNAGVSEEMIGVALAENGRRQKALIATKVRFRMGNGPNEVGLSRHHIIAQAEASLKRLKTDVIELYQVHEWDGMTPIEDTMEALDTLVKQGKVRYIACSNYSGWHIMKGLAAADKSHGQRFISQQIHYTLHSREAEYELVPISQDQGLGILIWSPLAGGLLSGKYRRDGGPDSGRHVGGSREPPVPDWDKLYEILDVIVAIAEERGVSGAQVALAWALGRPGVTSAIIGGRSEAQFRDNLGAADLKLSDEERQRLDAASRPPLLYPYWHQSFTANDRLGPADQDLIGTYAEDFKRG

SEQ ID NO: 80 - protein, 353 aa, Artificial Sequence
  enzyme
MDYRYLGRSGLRVSTLTMGTMTFAGSEKVGHTGQADATRQIDLCLDHGINLLDTANVYNAGVSEEMIGVGLSENGRRQKALIATKVRFRMANGPNEVGLSRHHIIAQAEASIKRLKTDVIDLYQVHEWDGMTPIDETMEALDTLVKQGKVRYIACSNYSGWHIMKGLAGADKSHGQRFISQQIHYTLHSREAEYELVPISQDQGLAILIWSPLAGGLLSGKYRRDGGPDSGRHVGGSREPPVPDWDKLYDILDVIVAIAEERGVSGAQVALAWALGRPGVTSAIIGGRSEAQFRDNLAAADLKLSDDERQRLDAASRPPLLYPYWHQTFTGQDRLDPADLDLLGTYAEEFKRG

SEQ ID NO: 81 - protein, 353 aa, Artificial Sequence
  enzyme
MDYRYLGRSGLRVSTLTMGTMTFGGSEKVGHTGQADATRQIDICLDHGINLLDTANVYNAGVSEEMLGVGLSENGRRQKALIATKVRFRMANGPNEVGLSRHHIIAQAEASIKRLKTDVIDLYQVHEWDGMTPIEDTMEALDTLVKQGKVRYIACSNYSGWHIMKALAGADKSHGQRFISQQIHYTLHSREAEYELVPISQDQGLGILIWSPLAGGLLSGKYRRDGGPDSGRHVGGSREPPVPDWDKLYDIIDVIVAIAEERGVSGAQVALAWALGRPGVTSAIIGGRSEAQFRDNLGAADLKLTDEERQRLDAASRPPLLYPYWHQTFTANDRLDPADLDLLSTYVEDFKRG

SEQ ID NO: 82 - protein, 353 aa, Artificial Sequence
  enzyme
MDYRYLGRSGLRVSTLTMGTMTFGGSEKVGHTGQADATRQLDLCLDHGINLLDTANVYNAGVSEEMIGVGLSENGRRQKALIATKVRFRMGNGPNEVGLSRHHIIAQAEASLKRLKTDVIELYQVHEWDGMTPIEDTMEALDTLVKQAKVRYIACSNYSGWHIMKALAGADKSHGQRFISQQIHYTLHSREAEYELVPISQDQGLAILIWSPLAGGLLSGKYRRDGGPDSGRHVGGSREPPVPDWDKLYEIIDVIVAIAEERGVSGAQVALAWALGRPGVTSAIIGGRSEAQFRDNLAAADLKLTDEERQRLDAASRPPLLYPYWHQTFTAQDRLGPADQDLIGTYAEDFKRG

SEQ ID NO: 83 - protein, 353 aa, Artificial Sequence
  enzyme
MDYRYLGRSGIRVSTLTMGTMTFGGSEKVGHTAQADATRQLDLCLDHGINLLDTANVYNAGVSEEMIGVALSENGRRQKALIATKVRFRMANGPNEVGLSRHHIIAQAEASIKRLKTDVIELYQVHEWDGMTPIEETMEALDTLVKQAKVRYIGCSNYSGWHIMKALAGADKSHGQRFISQQIHYTLHSREAEYELVPISQDQGLGILIWSPLAGGLLSGKYRRDGGPDSGRHVGGSREPPVPDWDKLYDIIDVIVAIAEERGVSGAQVALAWALGRPGVTSAIIGGRSEAQFRDNLGAADLKLTDEERQRLDAASRPPLLYPYWHQSFTGNDRLDPADLDLLGTYADEFKRG

SEQ ID NO: 84 - protein, 353 aa, Artificial Sequence
  enzyme
MDYRYLGRSGIRVSTLTMGTMTFAGSEKVGHTAQADATRQLDICLDHGINLLDTANVYNAGVSEEMLGVGLSENGRRQKALIATKVRFRMANGPNEVGLSRHHIIAQAEASLKRLKTDVIELYQVHEWDGMTPIDETMEALDTLVKQAKVRYIACSNYSGWHIMKGLAGADKSHGQRFISQQIHYTLHSREAEYELVPISQDQGLGILIWSPLAGGLLSGKYRRDGGPDSGRHVGGSREPPVPDWDKLYEIIDVIVAIAEERGVSGAQVALAWALGRPGVTSAIIGGRSEAQFRDNLGAADLKLSDEERQRLDAASRPPLLYPYWHNSFTGNDRLDPADLDLLGTYADEFKRG

SEQ ID NO: 85 - protein, 353 aa, Artificial Sequence
  enzyme
MDYRYLGRSGLRVSTLTMGTMTFGGSDKVGHTPQADATRQIDICLDHGINLLDTANVYNAGVSEEMIGVALAEGRRQQKALIATKVRFRGGGGPNEVGLSKHHIIAQAEASLKRLKTDVIELYQVHEWDGMTPIEETMEALDTLVKQGKVRYIACSNYSGWHIMKALAAADKSHGQRFISQQIHYTLHSREADYELVPISQDQGLGILIWSPLAGGLLSGKYRRDGGPDAGRHVGGSREPPVPDWDKLYEIIDVIVAIAEERGVSGAQVALAWALGRPGVTSAIIGGRSEAQFRDNLAAAELKLTDDERQRLDAASRPPLLYPYWHQSFTAQERLGPADQDLLSTYVEDFKRG

SEQ ID NO: 86 - protein, 353 aa, Artificial Sequence
  enzyme
MDYKYLGRSGLRVSTLTMGTMTFGGSEKVGHTPQADATRQIDLCLDHGINLLDTANVYNAGVSEEMIGVALAEHGRRQKALIATKVRFRMGDGPNEVGLSRHHIIAQAEASLKRLKTDVIDLYQVHEWDGMTPIEETMEALDTLVKQGKVRYIGCSNYSGWHIMKALAAADKSHGQRFISQQIHYTLHSREAEYELVPISQDQGLGILIWSPLAGGLLSGKYRRDGGPDAGRHVGGSRDPPVPDWDKLYEILDVIVAIAREKDVSGAQVALAWALGRPGVTSAIIGGRSEAQFRDNLAAAELKLTDDERQRLDAASRPPLLYPYWHQSFTGQDRLDQVDLDLIGPYAEEFKRG

SEQ ID NO: 87 - protein, 353 aa, Artificial Sequence
  enzyme
MDYKYLGRSGIRVSTLTMGTMTFGGSEKVGHTPQADATRQIDLCLDHGINLLDTANVYNAGVSEEMIGVALAEHGRRQKALIATKVRFRMGDGPNEVGLSRHHIIAQAEASLKRIKTDVIDLYQVHEWDGMTPIEETMEALDTLVKQAKVRYIGCSNYSGWHIMKALAGADKSHGQRFISQQIHYTLHSREAEYELVPISQDQGLGILIWSPLAGGLLSGKYRRDGGPDAGRHVGGSRDPPVPDWDRLYDIIDVIVAIAEERGVSGAQVALAYALGRPGVTSAIIGGRSEAQFRDNLGAAELKLTDDERQRLDAASRPPLLYPYWHNSFTGQDRLGPADQDLIGPYAEEFKRG

SEQ ID NO: 88 - protein, 353 aa, Artificial Sequence
  enzyme
MDYRYLGRSGIRVSTLTMGTMTFGGSEKVGHTPQADATRQIDICLDHGINLLDTANVYNAGVSEEMIGVALAEHGRRQKALIATKVRFRMGDGPNEVGLSRHHIIAQAEASLKRIKTDVIDLYQVHEWDGMTPIEETMEALDTLVKQGKVRYIGCSNYSGWHIMKALAAADKSHGQRFISQQIHYTLHSREGEYELVPISQDQGLAILIWSPLAGGLLSGKYKRDGGPDAGRHVGGSREPPLPDWDRLYDIIDVIVAIARERDVSGAQVALAFALGRPGVTSAIIGGRSEANFRDNLGAAELKLSDDERQRLDAASRPPLLYPYWHQSFTANDRLDQLDLDLIGPYADEFKRG

SEQ ID NO: 89 - protein, 353 aa, Artificial Sequence
  enzyme
MDYRYIGRSGLKVSAMTMGTMTFGGSERVGHTDLAGAARQVDLCLDAGINLYDTANVYNAGVSEDILGQVLAEHGRRQRALVATKVRFRMGNGPNEAGLSKHHIIAQAEASLKRLRTDAIELYQVHEWDGMTPIEETMEALDTLVRQGKVRYVGCSNYSGWHIMKALMAADKHHGQRFVSQQIHYSLHSRDAEYELVPISQDQGLGILVWSPLAGGLLSGKYRRTGGPEAGRHVGGFREPPVYDWDKLYELIDVIVAIAAQRGVSGAQVALAWLLGRPGVTSLIIGGRSEAQFRDNLAAAHLRLTSEERARLDAASRPPLLYPYWHQSFTAQDRLSRIDLDLIGPYAEEFKRG

SEQ ID NO: 90 - protein, 353 aa, Artificial Sequence
  enzyme
MDYRYLGRSGLKVSAMTMGTMTFGGSERVGHTDLAGAARQIDLCIDAGINLLDTANVYNAGVSEDIIGVALAEHGRRQRALVATKVRFKMGNGPNEVGLSRHHIIAQAEASLKRLRTDAIDLYQVHEWDGMTPIEETMEALDTLVKQGKVRYVGCSNYSGWHIMKALMAADKRQGQRFISQQIHYSLHSREAEYELVPISQDQGLGILIWSPLAGGLLSGKYRRDGGPESGRHVGGFREPPVYDWDKLYEIIDVIVAIARQKGVSGAQVALSWLLERPGVTSLIIGGRSEAQFADNLAAIHLRLTSDERARLDAASRPPLLYPYWHQSFTAQDRLSQIDLDLIGPYAEEFKRG

SEQ ID NO: 91 - protein, 353 aa, Artificial Sequence
  enzyme
MDYRYLGRSGLKVSAMTMGTMTFGGSERVGHTDLAGAARQIDLCLDHGINLYDTANVYNAGVSEDIIGQALAEHGRRQRALIATKVRFKMGNGPNEAGLSRHHIIAQAEASLKRLRTDAIELYQVHEWDGMTPIEETMEALDTLVKQAKVRYVGCSNYSGWHIMKALAAADKRQGQRFISQQIHYSLHSRDAEYELVPISQDQGLGILIWSPLAGGLLSGKYRRDGGPESGRHVGGFREPPVYDWDRLYDLIDVIVDIAAQKGVSGAQVALSYALGRPGVTSLIIGGRNEAQFRDNLAAIHLKLTDEERARLDAASRPPLLYPYWHQSFTAQDRLSRIVDLDLEPYAEEFKRG

SEQ ID NO: 92 - protein, 353 aa, Artificial Sequence
  enzyme
MDYRFLGRSGLKVSAMTMGTMTFGGSERVGHTAQAGAARQVDLCLDAGINLLDTANVYNAGVSEDILGVVLAEHGRRQRALVATKVRFKMGNGPNEAGLSRHHIIAQAEASLKRLRTDAIDLYQVHEWDGMTPIDETMEALDTLVRQGKVRYVGCSNYSGWHIMKALMAADKRQGQRFVSQQIHYSLHSRDAEYELVPISQDQGLGILVWSPLAGGLLSGKYKRDGGPESGRHVGGFREPPLYDWDKLYDLIDVIVAIARQRGVSGAQVALSFLLERPGVTSLIIGGRSEANFADNLAAAHLKLSSEERARLDAASRPPLLYPYWHQSFTAQDRLSQIDLDLIEPYAEEFKRG

SEQ ID NO: 93 - protein, 353 aa, Artificial Sequence
  enzyme
MDYKYIGRSGLKVSAMTMGTMTFGGSERVGHTDLAGAARQVDICLDAGINLLDTANVYNAGVSEDILGVVLAEHGRRQRALIATKVRFRMGNGPNEGGLSRHHIIAQAEASLKRLRTDAIELYQVHEWDGMTPIDETMEALDTLVKQAKVRYVACSNYSGWHIMKALAGADKRQGQRFVSQQIHYSLHSRDGEYELVPISQDQGLGILIWSPLAGGLLSGKYRRDGGPESGRHVGGFREPPVYDWDKLYEIIDVIVDIARQRGVSGAQVALAWALERPGVTSLIIGGRSEAQFADNIAAIHLKLSDEERARLDAASRPPLLYPYWHQSFTGQDRLSQIDLDLIEPYAEEFKRG

SEQ ID NO: 94 - protein, 353 aa, Artificial Sequence
  enzyme
MDYKYLGRSGLKVSAMTMGTMTFGGSERVGHTGQAGATRQVDICLDAGINLLDTANVYNAGVSEEMLGVVLAEHGRRQRALIATKVRFKMGNGPNEVGLSRHHIIAQAEASLKRLRTDVIELYQVHEWDGMTPIEDTMEALDTLVRQAKVRYVGCSNYSGWHIMKGLAGADKRQGQRFISQQIHYTLHSRDAEYELVPISQDQGLGILIWSPLAGGLLSGKYRRDGGPDAGRHVGGFREPPVYDWDKLYELIDVIVDIARQRGVSGAQVALSWALERPGVTSLIIGGRSEAQFADNIAGAHLKLSSEERARLDAASRPPLLYPYWHQSFTGQDRLSQIDLDLIGPYAEEFKRG

SEQ ID NO: 95 - protein, 353 aa, Artificial Sequence
  enzyme
MDYKYLGRSGLKVSAMTMGTMTFGGSERVGHTDLAGAARQVDLCLDAGINLYDTANVYNAGVSEDMLGVVLAENGRRQRALVATKVRFKMGNGPNEAGLSRHHIIAQAEASLKRLRTDAIDLYQVHEWDGMTPIDETMEALDTLVRQGKVRYVGCSNYSGWHIMKALMAADKRQGQRFVSQQIHYSLHSRDAEYELVPISQDQGLGILVWSPLAGGLLSGKYRRTGGPESGRHVGGFREPPVYDWDKLYDLIDVIVAIARQRGVSGAQVALAWLLERPGVTSLIIGGRSEAQFRDNIAAIHLKLSSEERARLDAASRPPLLYPYWHNSFTGQDRLDQIDLDLIEPYAEEFKRG

SEQ ID NO: 96 - protein, 353 aa, Artificial Sequence
  enzyme
MDYKYLGRSGLKVSAMTMGTMTFGGSERVGHTAQAGAARQVDLCLDHGINLLDTANVYNAGVSEEMLGVVLAEHGRRQKALVATKVRFKMGNGPNEGGLSRHHIIAQAEASLKRLKTDAIELYQVHEWDGMTPIEDTMEALDTLVRQGKVRYVACSNYSGWHIMKALAAADKRQGQRFVSQQIHYSLHSRDAEYELVPISQDQGLGILVWSPLAGGLLSGKYRRDGGPESGRHVGGFREPPVYDWDKLYEILDVIVAIARQRGVSGAQVALAWLLERPGVTSLIIGGRSEAQFADNIAAIHLKLSDEERARLDAASRPPLLYPYWHQSFTANDRLDQIDLDLIEPYAEDFKRG

SEQ ID NO: 97 - protein, 353 aa, Artificial Sequence
  enzyme
MDYRYLGRSGLKVSAMTMGTMTFGGSERVGHTDLAGATRQVDLCLDHGINLLDTANVYNAGVSEEMIGVVLSEHGRRQRALIATKVRFKMGNGPNEGGLSRHHIIAQAEASLKRLRTDAIDLYQVHEWDGMTPIDETMEALDTLVRQGKVRYVACSNYSGWHIMKALMGADKRQGQRFVSQQIHYTLHSRDGEYELVPISQDQGLGILVWSPLAGGLLSGKYRRDGGPDAGRHVGGFREPPVYDWDKLYDLLDVIVDIARQRGVSGAQVALSWLLGRPGVTSLIIGGRSEAQFRDNIAAAHLKLSSDERARLDAASRPPLLYPYWHQSFTAQDRLDQIDLDLLEPYAEEFKRG

SEQ ID NO: 98 - protein, 353 aa, Artificial Sequence
  enzyme
MDYRYIGRSGLKVSAMTMGTMTFGGSEKVGHTGQAGAARQVDLCLDHGINLLDTANVYNAGVSEDILGVVLAEHGRRQKALIATKVRFRMGNGPNEVGLSRHHIIAQAEASLKRLRTDAIDLYQVHEWDGMTPIEDTMEALDTLVRQGKVRYVACSNYSGWHIMKALAGADKHHGQRFISQQIHYTLHSREAEYELVPISQDQGLGILIWSPLAGGLLSGKYRRDGGPESGRHVGGFREPPVYDWDKLYDLIDVIVDIARQRGVSGAQVALSWLLERPGVTSLIIGGRSEAQFRDNIAAIHLKLTSEERARLDAASRPPLLYPYWHNSFTAQDRLSQIDLDLIGPYAEDFKRG

SEQ ID NO: 99 - protein, 353 aa, Artificial Sequence
  enzyme
MDYRYLGRSGLKVSAMTMGTMTFGGSERVGHTGQAGAARQLDLCLDAGINLLDTANVYNAGVSEDILGVVLSEHGRRQRALVATKVRFKMGNGPNEGGLSRHHIIAQAEASLKRLRTDVIELYQVHEWDGMTPIEDTMEALDTLVKQAKVRYVACSNYSGWHIMKALMGADKHHGQRFVSQQIHYSLHSRDAEYELVPISQDQGLGILIWSPLAGGLLSGKYRRDGGPDAGRHVGGFREPPVYDWDKLYELIDVIVAIARQRGVSGAQVALAWLLERPGVTSLIIGGRSEAQFRDNLAAAHLKLTDEERARLDAASRPPLLYPYWHQSFTAQDRLSQIDLDLIEPYAEDFKRG

SEQ ID NO: 100 - protein, 353 aa, Artificial Sequence
  enzyme
MDYRYIGRSGLKVSAMTMGTMTFGGSERVGHTDLAGATRQVDLCLDAGINLLDTANVYNAGVSEEMIGVVLAEHGRRQRALVATKVRFRMGNGPNEVGLSRHHIIAQAEASLKRLRTDAIELYQVHEWDGMTPIEETMEALDTLVRQAKVRYVGCSNYSGWHIMKALMGADKRQGQRFVSQQIHYSLHSRDGEYELVPISQDQGLGILVWSPLAGGLLSGKYRRDGGPDAGRHVGGFREPPVYDWDKLYDLIDVIVDIARQRGVSGAQVALAWALERPGVTSLIIGGRSEAQFADNLAAIHLKLTSEERARLDAASRPPLLYPYWHQSFTGNDRLDQIDLDLIGPYADEFKRG

SEQ ID NO: 101 - protein, 353 aa, Artificial Sequence
  enzyme
MDYRYIGRSGLKVSAMTMGTMTFGGSERVGHTAQAGAARQVDLCLDAGINLYDTANVYNAGVSEDILGVVLSENGRRQKALVATKVRFKMGNGPNEAGLSRHHIIAQAEASLKRLKTDAIDLYQVHEWDGMTPIEETMEALDTLVRQGKVRYVGCSNYSGWHIMKALMAADKRQGQRFVSQQIHYSLHSRDAEYELVPISQDQGLGILVWSPLAGGLLSGKYRRTGGPESGRHVGGFREPPVYDWDKLYELIDVIVDIAAQRGVSGAQVALAWLLGRPGVTSLIIGGRNEAQFRDNIAAIHLKLSSEERARLDAASRPPLLYPYWHQSFTGQDRLDQIDLDLIGPYADEFKRG